European Patent Application EP 4 218 745 A1, published August 2, 2023. Title: USE OF 2-PENTANONE AND SPECIFIC RECEPTOR THEREOF IN MANUFACTURE OF PRODUCTS REGULATING CELL FUNCTIONS. Applicant: Taihe Hospital, Hubei University of Medicine. The sequence listing filed with the application follows.

SEQUENCE LISTING (11 sequences)

SEQ ID NO: 1 - DNA, 1230 bp, synthetic construct
  misc_feature 1..1230: note = The sequence is synthetized.
  source 1..1230: mol_type = other DNA
atggttcgttacgtgccccggttcgctgatggtcagaaagtaaagttggcttggcccttggcggtttttcggttaaatcacatattctggccattggatccgagcacagggaaatggggccgatatctggacaaggttctagctgttgcgatgtccttggtttttatgcaacacaacgatgcagagctgaggtacttgcgcttcgaggcaagtaatcggaatttggatgcctttctcacaggaatgccaacgtatttaatcctcgtggaggctcaatttagaagtcttcacattctactgcacttcgagaagcttcagaagtttttagaaatattctacgcaaatatttatattgatccccgtaaggaacccgaaatgtttcgaaaagtggatggaaagatgataattaacagattagtttcggccatgtacggtgcagttatctctctgtatctaatcgcacccgttttttccatcattaaccaaagcaaagattttctatactctatgatctttccgttcgattcggatcccttgtacatatttgtgccactgcttttgacaaacgtatgggttggcattgtaatagataccatgatgttcggggagacgaatttgttgtgtgaactaattgtccacctaaatggtagttatatgttgctcaagagggacttgcagttggccattgaaaagatattagttgcaagggaccgtccgcatatggccaaacagctaaaggttttaattacaaaaactctccgaaagaatgtggctctaaatcagtttggccagcagctggaggctcagtatactgtgcgggtttttattatgtttgcattcgctgcgggccttttatgtgctctttcttttaaggcttatacgaatcctatggctaattacatctatgcgatttggtttggtgctaagacagttgagctgctttctttaggacagattggttccgacttggcctttactacggattccctcagcacaatgtactaccttacccattgggagcaaatcctgcagtactctacaaatcccagcgaaaatctgcgattactaaagctcattaacttggccattgagatgaacagcaagcccttctatgtgacagggctaaaatattttcgcgttagtctgcaggctggcttaaaaattctgcaggcatccttctcgtacttcacattcctcacttcgatgcagcgacgacaaatgagcaattaa

SEQ ID NO: 2 - DNA, 1461 bp, synthetic construct
  misc_feature 1..1461: note = The sequence is synthetized.
  source 1..1461: mol_type = other DNA
atgacaacctcgatgcagccgagcaagtacacgggcctggtcgccgacctgatgcccaacatccgggcgatgaagtactccggcctgttcatgcacaacttcacgggcggcagtgccttcatgaagaaggtgtactcctccgtgcacctggtgttcctcctcatgcagttcaccttcatcctggtcaacatggccctgaacgccgaggaggtcaacgagctgtcgggcaacacgatcacgaccctcttcttcacccactgcatcacgaagtttatctacctggctgttaaccagaagaatttctacagaacattgaatatatggaaccaggtgaacacgcatcccttgttcgccgagtcggatgctcgttaccattcgatcgcactggcgaagatgaggaagctgttctttctggtgatgctgaccacagtcgcctcggccaccgcctggaccacgatcaccttctttggcgacagcgtaaaaatggtggtggaccatgagacgaactccagcatcccggtggagataccccggctgccgattaagtccttctacccgtggaacgccagccacggcatgttctacatgatcagctttgcctttcagatctactacgtgctcttctcgatgatccactccaatctatgcgacgtgatgttctgctcttggctgatattcgcctgcgagcagctgcagcacttgaagggcatcatgaagccgctgatggagctgtccgcctcgctggacacctacaggcccaactcggcggccctcttcaggtccctgtcggccaactccaagtcggagctaattcataatgaagaaaaggatcccggcaccgacatggacatgtcgggcatctacagctcgaaagcggattggggcgctcagtttcgagcaccctcgacactgcagtcctttggcgggaacgggggcggaggcaacgggttggtgaacggcgctaatcccaacgggctgaccaaaaagcaggagatgatggtgcgcagtgccatcaagtactgggtcgagcggcacaagcacgtggtgcgactggtggctgccatcggcgatacttacggagccgccctcctcctccacatgctgacctcgaccatcaagctgaccctgctggcataccaggccaccaaaatcaacggagtgaatgtctacgccttcacagtcgtcggatacctaggatacgcgctggcccaggtgttccacttttgcatctttggcaatcgtctgattgaagagagttcatccgtcatggaggccgcctactcgtgccactggtacgatggctccgaggaggccaagaccttcgtccagatcgtgtgccagcagtgccagaaggcgatgagcatatcgggagcgaaattcttcaccgtctccctggatttgtttgcttcggttctgggtgccgtcgtcacctactttatggtgctggtgcagctcaagtaa

SEQ ID NO: 3 - protein, 933 aa, synthetic construct
  REGION 1..933: note = The sequence is synthetized.
MVRYVPRFADGQKVKLAWPLAVFRLNHIFWPLDPSTGKWGRYLDKVLAVAMSLVFMQHNDAELRYLRFEASNRNLDAFLTGMPTYLILVEAQFRSLHILLHFEKLQKFLEIFYANIYIDPRKEPEMFRKVDGKMIINRLVSAMYGAVISLYLIAPVFSIINQSKDFLYSMIFPFDSDPLYIFVPLLLTNVWVGIVIDTMMFGETNLLCELIVHLNGSYMLLKRDLQLAIEKILVARDRPHMAKQLKVLITKTLRKNVALNQFGQQLEAQYTVRVFIMFAFAAGLLCALSFKAYTNPMANYIYAIWFGAKTVELLSLGQIGSDLAFTTDSLSTMYYLTHWEQILQYSTNPSENLRLLKLINLAIEMNSKPFYVTGLKYFRVSLQAGLKILQASFSYFTFLTSMQRRQMSNATNFSLLKQAGDVEENPGPMTTSMQPSKYTGLVADLMPNIRAMKYSGLFMHNFTGGSAFMKKVYSSVHLVFLLMQFTFILVNMALNAEEVNELSGNTITTLFFTHCITKFIYLAVNQKNFYRTLNIWNQVNTHPLFAESDARYHSIALAKMRKLFFLVMLTTVASATAWTTITFFGDSVKMVVDHETNSSIPVEIPRLPIKSFYPWNASHGMFYMISFAFQIYYVLFSMIHSNLCDVMFCSWLIFACEQLQHLKGIMKPLMELSASLDTYRPNSAALFRSLSANSKSELIHNEEKDPGTDMDMSGIYSSKADWGAQFRAPSTLQSFGGNGGGGNGLVNGANPNGLTKKQEMMVRSAIKYWVERHKHVVRLVAAIGDTYGAALLLHMLTSTIKLTLLAYQATKINGVNVYAFTVVGYLGYALAQVFHFCIFGNRLIEESSSVMEAAYSCHWYDGSEEAKTFVQIVCQQCQKAMSISGAKFFTVSLDLFASVLGAVVTYFMVLVQLKATNFSLLKQAGDVEENPGP

SEQ ID NO: 4 - protein, 409 aa, synthetic construct
  REGION 1..409: note = The sequence is synthetized.
MVRYVPRFADGQKVKLAWPLAVFRLNHIFWPLDPSTGKWGRYLDKVLAVAMSLVFMQHNDAELRYLRFEASNRNLDAFLTGMPTYLILVEAQFRSLHILLHFEKLQKFLEIFYANIYIDPRKEPEMFRKVDGKMIINRLVSAMYGAVISLYLIAPVFSIINQSKDFLYSMIFPFDSDPLYIFVPLLLTNVWVGIVIDTMMFGETNLLCELIVHLNGSYMLLKRDLQLAIEKILVARDRPHMAKQLKVLITKTLRKNVALNQFGQQLEAQYTVRVFIMFAFAAGLLCALSFKAYTNPMANYIYAIWFGAKTVELLSLGQIGSDLAFTTDSLSTMYYLTHWEQILQYSTNPSENLRLLKLINLAIEMNSKPFYVTGLKYFRVSLQAGLKILQASFSYFTFLTSMQRRQMSN

SEQ ID NO: 5 - protein, 486 aa, synthetic construct
  REGION 1..486: note = The sequence is synthetized.
MTTSMQPSKYTGLVADLMPNIRAMKYSGLFMHNFTGGSAFMKKVYSSVHLVFLLMQFTFILVNMALNAEEVNELSGNTITTLFFTHCITKFIYLAVNQKNFYRTLNIWNQVNTHPLFAESDARYHSIALAKMRKLFFLVMLTTVASATAWTTITFFGDSVKMVVDHETNSSIPVEIPRLPIKSFYPWNASHGMFYMISFAFQIYYVLFSMIHSNLCDVMFCSWLIFACEQLQHLKGIMKPLMELSASLDTYRPNSAALFRSLSANSKSELIHNEEKDPGTDMDMSGIYSSKADWGAQFRAPSTLQSFGGNGGGGNGLVNGANPNGLTKKQEMMVRSAIKYWVERHKHVVRLVAAIGDTYGAALLLHMLTSTIKLTLLAYQATKINGVNVYAFTVVGYLGYALAQVFHFCIFGNRLIEESSSVMEAAYSCHWYDGSEEAKTFVQIVCQQCQKAMSISGAKFFTVSLDLFASVLGAVVTYFMVLVQLK

SEQ ID NO: 6 - DNA, 27 bp, synthetic construct
  misc_feature 1..27: note = The sequence is synthetized.
  source 1..27: mol_type = other DNA
gctctagaatggttcgttacgtgcccc

SEQ ID NO: 7 - DNA, 78 bp, synthetic construct
  misc_feature 1..78: note = The sequence is synthetized.
  source 1..78: mol_type = other DNA
aggtccagggttctcctccacgtctccagcctgcttcagcaggctgaagttagtagcattgctcatttgtcgtcgctg

SEQ ID NO: 8 - DNA, 77 bp, synthetic construct
  misc_feature 1..77: note = The sequence is synthetized.
  source 1..77: mol_type = other DNA
gctactaacttcagcctgctgaagcaggctggagacgtggaggagaaccctggacctatgacaacctcgatgcagcc

SEQ ID NO: 9 - DNA, 83 bp, synthetic construct
  misc_feature 1..83: note = The sequence is synthetized.
  source 1..83: mol_type = other DNA
ccaccggtaggtccagggttctcctccacgtctccagcctgcttcagcaggctgaagttagtagccttgagctgcaccagcac

SEQ ID NO: 10 - DNA, 27 bp, synthetic construct
  misc_feature 1..27: note = The sequence is synthetized.
  source 1..27: mol_type = other DNA
gctctagaatggttcgttacgtgcccc

SEQ ID NO: 11 - DNA, 83 bp, synthetic construct; identical to SEQ ID NO: 9
  misc_feature 1..83: note = The sequence is synthetized.
  source 1..83: mol_type = other DNA